European Patent Application EP 4 386 000 A1, published June 19, 2024. Title: RECOMBINANT ANTI-HUMAN-CD25 ANTIBODY AND USE THEREOF. Applicant: Nanjing Novoacine Biotechnology Co., Ltd. The sequence listing filed with the application follows.

SEQUENCE LISTING (105 sequences)

SEQ ID NO: 1 - protein, 120 aa, artificial sequence
  REGION 1..120: note = 2046-2H1
DVQLQESGPGLVKPSQSLSLTCTVTGYSITSDYAWNWIRHFPGNKLEWMGYITYSGSTVYNPSLKSRISITRDTSKNHFFLQLNSVTTEDTATYYCARWLLQIYYAMDYWGQGTSVTVSS

SEQ ID NO: 2 - protein, 120 aa, artificial sequence
  REGION 1..120: note = 2046-2H1-HZ0
EVQLQESGPGLVKPSQTLSLTCTVSGYSITSDYAWNWIRQPPGKGLEWIGYITYSGSTVYNPSLKSRVTISVDTSKNQFSLKLSSVTAADTAVYYCARWLLQIYYAMDYWGQGTLVTVSS

SEQ ID NO: 3 - protein, 120 aa, artificial sequence
  REGION 1..120: note = 2046-2H1-HZ1
EVQLQESGPGLVKPSQTLSLTCTVSGYSITSDYAWNWIRQPPGKGLEWIGYITYSGSTVYNPSLKSRVTISRDTSKNQFSLKLSSVTAADTAVYYCARWLLQIYYAMDYWGQGTLVTVSS

SEQ ID NO: 4 - protein, 120 aa, artificial sequence
  REGION 1..120: note = 2046-18H1
DVQLQESGPGLVKPSQSLSLTCTVTGYSITSDYAWNWIRQFPGNKLEWMGYISYSGITIYNPSLKSRISITRDTSKNQFFLQLNSVTTEDTATYYCARWLLQIYYAMDYWGQGTSVTVSS

SEQ ID NO: 5 - protein, 120 aa, artificial sequence
  REGION 1..120: note = 2046-18H1-HZ0
EVQLQESGPGLVKPSQTLSLTCTVSGYSITSDYAWNWIRQPPGKGLEWIGYISYSGITIYNPSLKSRVTISVDTSKNQFSLKLSSVTAADTAVYYCARWLLQIYYAMDYWGQGTLVTVSS

SEQ ID NO: 6 - protein, 120 aa, artificial sequence
  REGION 1..120: note = 2046-18H1-HZ1
EVQLQESGPGLVKPSQTLSLTCTVSGYSITSDYAWNWIRQPPGKGLEWIGYISYSGITIYNPSLKSRVTISRDTSKNQFSLKLSSVTAADTAVYYCARWLLQIYYAMDYWGQGTLVTVSS

SEQ ID NO: 7 - protein, 120 aa, artificial sequence
  REGION 1..120: note = 2046-24H2
DVQLQESGPGLVKPSQSLSLTCTVTGYSITSDYAWNWIRQFPGNKLEWMGYISYGGTTIYNPSLKSRISITRDTSKNQFFLQLNSVTTEDTATYYCARWLLQNYYAMDYWGQGTSVTVSS

SEQ ID NO: 8 - protein, 120 aa, artificial sequence
  REGION 1..120: note = 2046-24H2-HZ0
EVQLQESGPGLVKPSQTLSLTCTVSGYSITSDYAWNWIRQPPGKGLEWIGYISYGGTTIYNPSLKSRVTISVDTSKNQFSLKLSSVTAADTAVYYCARWLLQNYYAMDYWGQGTLVTVSS

SEQ ID NO: 9 - protein, 120 aa, artificial sequence
  REGION 1..120: note = 2046-24H2-HZ1
EVQLQESGPGLVKPSQTLSLTCTVSGYSITSDYAWNWIRQPPGKGLEWIGYISYGGTTIYNPSLKSRVTISRDTSKNQFSLKLSSVTAADTAVYYCARWLLQNYYAMDYWGQGTLVTVSS

SEQ ID NO: 10 - protein, 115 aa, artificial sequence
  REGION 1..115: note = 2046-36H2
QIQLVQSGPELKKPGETVRISCKASGYTFTTAGMQWVQKMPGKGLKWIGWINTHSGVPKYAEDFKGRFAFSLETSASTAYLQISNLKNEDTATYFCASDYAFGYWGQGTLVTVSA

SEQ ID NO: 11 - protein, 115 aa, artificial sequence
  REGION 1..115: note = 2046-36H2-HZ0
EVQLVQSGSELKKPGASVKVSCKASGYTFTTAGMQWVRQAPGQGLEWMGWINTHSGVPKYAEDFKGRFVFSLDTSVSTAYLQISSLKAEDTAVYYCARDYAFGYWGQGTLVTVSS

SEQ ID NO: 12 - protein, 115 aa, artificial sequence
  REGION 1..115: note = 2046-36H2-HZ1
EIQLVQSGSELKKPGASVKVSCKASGYTFTTAGMQWVRQAPGQGLEWMGWINTHSGVPKYAEDFKGRFVFSLDTSVSTAYLQISSLKAEDTAVYYCASDYAFGYWGQGTLVTVSS

SEQ ID NO: 13 - protein, 120 aa, artificial sequence
  REGION 1..120: note = 2046-61H1
DVQLQESGPGLVKPSQSLSLTCTVTGYSITSDYAWNWIRQFPGNKLEWMGYISYSGGTIYNPSLKSRISITRDTSKNQFFLQLNSVTTEDTATYYCARWLLQNYYAMDYWGQGTSVTVSS

SEQ ID NO: 14 - protein, 120 aa, artificial sequence
  REGION 1..120: note = 2046-61H1-HZ0
EVQLQESGPGLVKPSQTLSLTCTVSGYSITSDYAWNWIRQPPGKGLEWIGYISYSGGTIYNPSLKSRVTISVDTSKNQFSLKLSSVTAADTAVYYCARWLLQNYYAMDYWGQGTLVTVSS

SEQ ID NO: 15 - protein, 120 aa, artificial sequence
  REGION 1..120: note = 2046-61H1-HZ1
EVQLQESGPGLVKPSQTLSLTCTVSGYSITSDYAWNWIRQPPGKGLEWIGYISYSGGTIYNPSLKSRVTISRDTSKNQFSLKLSSVTAADTAVYYCARWLLQNYYAMDYWGQGTLVTVSS

SEQ ID NO: 16 - protein, 120 aa, artificial sequence
  REGION 1..120: note = 2046-111H2
DVQLQESGPGLVKPSQSLSLTCTVTGHSITSDYAWNWIRQFPGNKLEWMGYISYSGSTIYNPSLKSRISITRDTSKNQFFLQLNSVTTEDTATYYCARWLLQNYYAMDYWGQGTSVTVSS

SEQ ID NO: 17 - protein, 120 aa, artificial sequence
  REGION 1..120: note = 2046-111H2-HZ0
EVQLQESGPGLVKPSQTLSLTCTVSGHSITSDYAWNWIRQPPGKGLEWIGYISYSGSTIYNPSLKSRVTISVDTSKNQFSLKLSSVTAADTAVYYCARWLLQNYYAMDYWGQGTLVTVSS

SEQ ID NO: 18 - protein, 120 aa, artificial sequence
  REGION 1..120: note = 2046-111H2-HZ1
EVQLQESGPGLVKPSQTLSLTCTVSGHSITSDYAWNWIRQPPGKGLEWIGYISYSGSTIYNPSLKSRVTISRDTSKNQFSLKLSSVTAADTAVYYCARWLLQNYYAMDYWGQGTLVTVSS

SEQ ID NO: 19 - protein, 114 aa, artificial sequence
  REGION 1..114: note = 2047-3H8
QVQLKQSGAELVKPGASVKMSCKTSGYTFTDYVISWVKQRTGQGLEWIGEIYPGSGSTYYNEKFKGKATLTADISSNTAYMQLSSLTSEDSAVYFCASINFDYWGHGTTLTVSS

SEQ ID NO: 20 - protein, 114 aa, artificial sequence
  REGION 1..114: note = 2047-3H8-HZ0
EVQLVQSGAEVKKPGATVKISCKVSGYTFTDYVISWVQQAPGKGLEWMGEIYPGSGSTYYNEKFKGRVTITADTSTDTAYMELSSLRSEDTAVYYCATINFDYWGQGTLVTVSS

SEQ ID NO: 21 - protein, 114 aa, artificial sequence
  REGION 1..114: note = 2047-3H8-HZ1
EVQLVQSGAEVKKPGATVKISCKTSGYTFTDYVISWVQQAPGKGLEWMGEIYPGSGSTYYNEKFKGRVTITADISTNTAYMELSSLRSEDTAVYYCASINFDYWGQGTLVTVSS

SEQ ID NO: 22 - protein, 118 aa, artificial sequence
  REGION 1..118: note = 2047-10H1
QVQLQQSGPELVRPGVSVKISCKGSGYTFTDYAMHWVKQSHAKSLEWIGVISTYNGNTNYNQKFKGKATMTVDKSSSTAYMELARLTSEDSAIYYCARSYGNYPFDYWGQGTTLTVSS

SEQ ID NO: 23 - protein, 118 aa, artificial sequence
  REGION 1..118: note = 2047-10H1-HZ0
EVQLVQSGAEVKKPGATVKISCKVSGYTFTDYAMHWVQQAPGKGLEWMGVISTYNGNTNYNQKFKGRVTITADTSTDTAYMELSSLRSEDTAVYYCATSYGNYPFDYWGQGTLVTVSS

SEQ ID NO: 24 - protein, 118 aa, artificial sequence
  REGION 1..118: note = 2047-10H1-HZ1
EVQLVQSGAEVKKPGATVKISCKGSGYTFTDYAMHWVQQAPGKGLEWMGVISTYNGNTNYNQKFKGRVTITVDKSTSTAYMELSSLRSEDTAVYYCARSYGNYPFDYWGQGTLVTVSS

SEQ ID NO: 25 - protein, 118 aa, artificial sequence
  REGION 1..118: note = 2047-10H1-HZ2
EVQLVQSGAEVKKPGATVKISCKGSGYTFTDYAMHWVQQAPGKGLEWMGVISTYSGNTNYNQKFKGRVTITVDKSTSTAYMELSSLRSEDTAVYYCARSYGNYPFDYWGQGTLVTVSS

SEQ ID NO: 26 - protein, 112 aa, artificial sequence
  REGION 1..112: note = 2046-2L1
DVVMTQTPLSLPVSLGDQASISCRSSQSLVHSNGNTYLHWYLQKPGQSPKLLIYKVSNRFSGVPDRFSGSGSGTDFTLKISRVEAEDLGVYFCSQSTHVPLTFGAGTKLELK

SEQ ID NO: 27 - protein, 112 aa, artificial sequence
  REGION 1..112: note = 2046-2L1-HZ0
DVVMTQSPLSLPVTLGQPASISCRSSQSLVHSNGNTYLHWFQQRPGQSPRRLIYKVSNRFSGVPDRFSGSGSGTDFTLKISRVEAEDVGVYYCSQSTHVPLTFGQGTKLEIK

SEQ ID NO: 28 - protein, 112 aa, artificial sequence
  REGION 1..112: note = 2046-2L1-HZ1
DVVMTQSPLSLPVTLGQPASISCRSSQSLVHSNGNTYLHWYQQRPGQSPRLLIYKVSNRFSGVPDRFSGSGSGTDFTLKISRVEAEDLGVYFCSQSTHVPLTFGQGTKLEIK

SEQ ID NO: 29 - protein, 112 aa, artificial sequence
  REGION 1..112: note = 2046-2L1-HZ2
DVVMTQSPLSLPVTLGQPASISCRSSQSLVHSSGNTYLHWYQQRPGQSPRLLIYKVSNRFSGVPDRFSGSGSGTDFTLKISRVEAEDLGVYFCSQSTHVPLTFGQGTKLEIK

SEQ ID NO: 30 - protein, 112 aa, artificial sequence
  REGION 1..112: note = 2046-18L1
DVVMTQTPLSLPVSLGDQASISCSSSQSLVHSNGNTYLHWYLHKPGQSPKLLIYKVSNRFSGVPDRFSGSGSGTDFTLKISRVEAEDLGVYFCSQSTHVPLTFGAGTKLELK

SEQ ID NO: 31 - protein, 112 aa, artificial sequence
  REGION 1..112: note = 2046-18L1-HZ0
DVVMTQSPLSLPVTLGQPASISCSSSQSLVHSNGNTYLHWFQQRPGQSPRRLIYKVSNRFSGVPDRFSGSGSGTDFTLKISRVEAEDVGVYYCSQSTHVPLTFGQGTKLEIK

SEQ ID NO: 32 - protein, 112 aa, artificial sequence
  REGION 1..112: note = 2046-18L1-HZ1
DVVMTQSPLSLPVTLGQPASISCSSSQSLVHSNGNTYLHWYQQRPGQSPRLLIYKVSNRFSGVPDRFSGSGSGTDFTLKISRVEAEDLGVYFCSQSTHVPLTFGQGTKLEIK

SEQ ID NO: 33 - protein, 112 aa, artificial sequence
  REGION 1..112: note = 2046-18L1-HZ2
DVVMTQSPLSLPVTLGQPASISCSSSQSLVHSSGNTYLHWYQQRPGQSPRLLIYKVSNRFSGVPDRFSGSGSGTDFTLKISRVEAEDLGVYFCSQSTHVPLTFGQGTKLEIK

SEQ ID NO: 34 - protein, 112 aa, artificial sequence
  REGION 1..112: note = 2046-18L1-T2
EIVLTQSPGTLSLSPGERATLSCSSSQSLVHSNGNTYLHWYQQKPGQAPRLLIYKVSNRFSGIPDRFSGSGSGTDFTLTISRLEPEDFAVYYCSQSTHVPLTFGQGTKLEIK

SEQ ID NO: 35 - protein, 112 aa, artificial sequence
  REGION 1..112: note = 2046-24L1
DVVMTQTPLSLPVSLGDQASISCRSSQSLVHSNGNTYLHWYLQKPGQSPKVLIYKVSNRFSGVPDRFSGSGSGTDFTLKISRVEAEDLGVYFCSQNTHVPLTFGAGTKLELK

SEQ ID NO: 36 - protein, 112 aa, artificial sequence
  REGION 1..112: note = 2046-24L1-HZ0
DVVMTQSPLSLPVTLGQPASISCRSSQSLVHSNGNTYLHWFQQRPGQSPRRLIYKVSNRFSGVPDRFSGSGSGTDFTLKISRVEAEDVGVYYCSQNTHVPLTFGQGTKLEIK

SEQ ID NO: 37 - protein, 112 aa, artificial sequence
  REGION 1..112: note = 2046-24L1-HZ1
DVVMTQSPLSLPVTLGQPASISCRSSQSLVHSNGNTYLHWYQQRPGQSPRVLIYKVSNRFSGVPDRFSGSGSGTDFTLKISRVEAEDLGVYFCSQNTHVPLTFGQGTKLEIK

SEQ ID NO: 38 - protein, 112 aa, artificial sequence
  REGION 1..112: note = 2046-24L1-HZ2
DVVMTQSPLSLPVTLGQPASISCRSSQSLVHSSGNTYLHWYQQRPGQSPRVLIYKVSNRFSGVPDRFSGSGSGTDFTLKISRVEAEDLGVYFCSQNTHVPLTFGQGTKLEIK

SEQ ID NO: 39 - protein, 112 aa, artificial sequence
  REGION 1..112: note = 2046-36L1
DVVMTQTPLTLSVTIGQPASISCKSSQSLLYSNGKTYLYWLFQRPGQSPKRLIYLVSKLDSGVPDRFTGSGSGTDFTLKISRVEAEDLGVYYCVQGTHFPYTFGGGTKLEIK

SEQ ID NO: 40 - protein, 112 aa, artificial sequence
  REGION 1..112: note = 2046-36L-HZ0
DVVMTQSPLSLPVTLGQPASISCKSSQSLLYSNGKTYLYWFQQRPGQSPRRLIYLVSKLDSGVPDRFSGSGSGTDFTLKISRVEAEDVGVYYCVQGTHFPYTFGQGTKLEIK

SEQ ID NO: 41 - protein, 112 aa, artificial sequence
  REGION 1..112: note = 2046-36L-HZ1
DVVMTQSPLSLPVTLGQPASISCKSSQSLLYSNGKTYLYWLQQRPGQSPRRLIYLVSKLDSGVPDRFSGSGSGTDFTLKISRVEAEDLGVYYCVQGTHFPYTFGQGTKLEIK

SEQ ID NO: 42 - protein, 112 aa, artificial sequence
  REGION 1..112: note = 2046-36L-HZ2
DVVMTQSPLSLPVTLGQPASISCKSSQSLLYSSGKTYLYWLQQRPGQSPRRLIYLVSKLDSGVPDRFSGSGSGTDFTLKISRVEAEDLGVYYCVQGTHFPYTFGQGTKLEIK

SEQ ID NO: 43 - protein, 112 aa, artificial sequence
  REGION 1..112: note = 2046-36L-HZ3
DVVMTQSPLSLPVTLGQPASISCKSSQSLLYSSGKTYLYWLQQRPGQSPRRLIYLVSKLDAGVPDRFSGSGSGTDFTLKISRVEAEDLGVYYCVQGTHFPYTFGQGTKLEIK

SEQ ID NO: 44 - protein, 112 aa, artificial sequence
  REGION 1..112: note = 2046-61L2
DVVMTQTPLSLPVSLGDQASISCRSSQSLVHSNGNTYLHWNLQKPGQSPKLLIYKVSNRFSGVPDRFSGSGSGTDFTLKISRVEAEDLGVYFCSQSTHVPLTFSAGTKLELK

SEQ ID NO: 45 - protein, 112 aa, artificial sequence; identical to SEQ ID NO: 27
  REGION 1..112: note = 2046-61L2-HZ0

SEQ ID NO: 46 - protein, 112 aa, artificial sequence
  REGION 1..112: note = 2046-61L2-HZ1
DVVMTQSPLSLPVTLGQPASISCRSSQSLVHSNGNTYLHWNQQRPGQSPRLLIYKVSNRFSGVPDRFSGSGSGTDFTLKISRVEAEDLGVYFCSQSTHVPLTFGQGTKLEIK

SEQ ID NO: 47 - protein, 112 aa, artificial sequence
  REGION 1..112: note = 2046-61L2-HZ2
DVVMTQSPLSLPVTLGQPASISCRSSQSLVHSSGNTYLHWNQQRPGQSPRLLIYKVSNRFSGVPDRFSGSGSGTDFTLKISRVEAEDLGVYFCSQSTHVPLTFGQGTKLEIK

SEQ ID NO: 48 - protein, 112 aa, artificial sequence
  REGION 1..112: note = 2046-111L1
DVVMTQTPLSLPVSLGDQASISCRSSQSLVHSNGNTYLHWYLRKPGQSPKLLIYKVSNRFSGVPDRFSGSGSGTDFTLKISRVEAEDLGVYFCSQSTHVPLTFGAGTKLELK

SEQ ID NO: 49 - protein, 112 aa, artificial sequence; identical to SEQ ID NO: 27
  REGION 1..112: note = 2046-111L1-HZ0

SEQ ID NO: 50 - protein, 112 aa, artificial sequence; identical to SEQ ID NO: 28
  REGION 1..112: note = 2046-111L1-HZ1

SEQ ID NO: 51 - protein, 112 aa, artificial sequence; identical to SEQ ID NO: 29
  REGION 1..112: note = 2046-111L1-HZ2

SEQ ID NO: 52 - protein, 112 aa, artificial sequence
  REGION 1..112: note = 2046-111L1-T1
EIVLTQSPGTLSLSPGERATLSCRSSQSLVHSNGNTYLHWYQQKPGQAPRLLIYKVSNRFSGIPDRFSGSGSGTDFTLTISRLEPEDFAVYYCSQSTHVPLTFGQGTKLEIK

SEQ ID NO: 53 - protein, 107 aa, artificial sequence
  REGION 1..107: note = 2047-3L2
DIVMTQSPATLSVTPGDRVSLSCRASQSISDYLHWYQQKSHESPRLLIKYASQSISGIPSRFSGSGSGSDFTLSINSVEPEDVGVYYCQNGHSFPYTFGGGTKLEIK

SEQ ID NO: 54 - protein, 107 aa, artificial sequence
  REGION 1..107: note = 2047-3L2-HZ0
EIVMTQSPATLSLSPGERATLSCRASQSISDYLHWYQQKPGQAPRLLIYYASQSISGIPARFSGSGSGTDFTLTISSLQPEDFAVYYCQNGHSFPYTFGQGTKLEIK

SEQ ID NO: 55 - protein, 107 aa, artificial sequence
  REGION 1..107: note = 2047-3L2-HZ1
EIVMTQSPATLSLSPGERATLSCRASQSISDYLHWYQQKPGQAPRLLIKYASQSISGIPARFSGSGSGSDFTLTISSLQPEDVAVYYCQNGHSFPYTFGQGTKLEIK

SEQ ID NO: 56 - protein, 107 aa, artificial sequence
  REGION 1..107: note = 2047-3L2-HZ2
EIVMTQSPATLSLSPGERATLSCRASQSISDYLHWYQQKPGQAPRLLIKYASQSISGIPARFSGSGSGSDFTLTISSLQPEDVAVYYCQSGHSFPYTFGQGTKLEIK

SEQ ID NO: 57 - protein, 107 aa, artificial sequence
  REGION 1..107: note = 2047-3L2-HZ3
EIVMTQSPATLSLSPGERATLSCRASQSISDYLHWYQQKPGQAPRLLIKYASQSISGIPARFSGSGSGSDFTLTISSLQPEDVAVYYCQNAHSFPYTFGQGTKLEIK

SEQ ID NO: 58 - protein, 107 aa, artificial sequence
  REGION 1..107: note = 2047-10L2
DIKMTQSPSSMYASLGERVTITCKASQDINSYLSWFQQKPGKSPKTLIYRANRLVDGVPSRFSGSGSGQDYSLTISSLEYEDMGIYYCLQYDEFPYTFGGGTKLEIK

SEQ ID NO: 59 - protein, 107 aa, artificial sequence
  REGION 1..107: note = 2047-10L2-HZ0
DIQMTQSPSSLSASVGDRVTITCKASQDINSYLSWFQQKPGKAPKSLIYRANRLVDGVPSRFSGSGSGTDFTLTISSLQPEDFATYYCLQYDEFPYTFGQGTKLEIK

SEQ ID NO: 60 - protein, 107 aa, artificial sequence
  REGION 1..107: note = 2047-10L2-HZ1
DIQMTQSPSSLSASVGDRVTITCKASQDINSYLSWFQQKPGKAPKTLIYRANRLVDGVPSRFSGSGSGQDYTLTISSLQPEDMATYYCLQYDEFPYTFGQGTKLEIK

SEQ ID NO: 61 - protein, 107 aa, artificial sequence
  REGION 1..107: note = 2047-10L2-HZ2
DIQMTQSPSSLSASVGDRVTITCKASQDITSYLSWFQQKPGKAPKTLIYRANRLVDGVPSRFSGSGSGQDYTLTISSLQPEDMATYYCLQYDEFPYTFGQGTKLEIK

SEQ ID NO: 62 - protein, 107 aa, artificial sequence
  REGION 1..107: note = 2047-10L2-HZ3
DIQMTQSPSSLSASVGDRVTITCKASQDITSYLSWFQQKPGKAPKTLIYRANRLVSGVPSRFSGSGSGQDYTLTISSLQPEDMATYYCLQYDEFPYTFGQGTKLEIK

SEQ ID NO: 63 - protein, 11 aa, artificial sequence
  REGION 1..11: note = HCDR1
GYSITSDYAWN

SEQ ID NO: 64 - protein, 16 aa, artificial sequence
  REGION 1..16: note = HCDR2
YITYSGSTVYNPSLKS

SEQ ID NO: 65 - protein, 11 aa, artificial sequence
  REGION 1..11: note = HCDR3
WLLQIYYAMDY

SEQ ID NO: 66 - protein, 16 aa, artificial sequence
  REGION 1..16: note = HCDR2
YISYSGITIYNPSLKS

SEQ ID NO: 67 - protein, 16 aa, artificial sequence
  REGION 1..16: note = HCDR2
YISYGGTTIYNPSLKS

SEQ ID NO: 68 - protein, 11 aa, artificial sequence
  REGION 1..11: note = HCDR3
WLLQNYYAMDY

SEQ ID NO: 69 - protein, 10 aa, artificial sequence
  REGION 1..10: note = HCDR1
GYTFTTAGMQ

SEQ ID NO: 70 - protein, 17 aa, artificial sequence
  REGION 1..17: note = HCDR2
WINTHSGVPKYAEDFKG

SEQ ID NO: 71 - protein, 6 aa, artificial sequence
  REGION 1..6: note = HCDR3
DYAFGY

SEQ ID NO: 72 - protein, 16 aa, artificial sequence
  REGION 1..16: note = HCDR2
YISYSGGTIYNPSLKS

SEQ ID NO: 73 - protein, 11 aa, artificial sequence
  REGION 1..11: note = HCDR1
GHSITSDYAWN

SEQ ID NO: 74 - protein, 16 aa, artificial sequence
  REGION 1..16: note = HCDR2
YISYSGSTIYNPSLKS

SEQ ID NO: 75 - protein, 10 aa, artificial sequence
  REGION 1..10: note = HCDR1
GYTFTDYVIS

SEQ ID NO: 76 - protein, 17 aa, artificial sequence
  REGION 1..17: note = HCDR2
EIYPGSGSTYYNEKFKG

SEQ ID NO: 77 - protein, 5 aa, artificial sequence
  REGION 1..5: note = HCDR3
INFDY

SEQ ID NO: 78 - protein, 10 aa, artificial sequence
  REGION 1..10: note = HCDR1
GYTFTDYAMH

SEQ ID NO: 79 - protein, 17 aa, artificial sequence
  REGION 1..17: note = HCDR2
VISTYNGNTNYNQKFKG

SEQ ID NO: 80 - protein, 9 aa, artificial sequence
  REGION 1..9: note = HCDR3
SYGNYPFDY

SEQ ID NO: 81 - protein, 17 aa, artificial sequence
  REGION 1..17: note = HCDR2
VISTYSGNTNYNQKFKG

SEQ ID NO: 82 - protein, 16 aa, artificial sequence
  REGION 1..16: note = LCDR1
RSSQSLVHSNGNTYLH

SEQ ID NO: 83 - protein, 7 aa, artificial sequence
  REGION 1..7: note = LCDR2
KVSNRFS

SEQ ID NO: 84 - protein, 9 aa, artificial sequence
  REGION 1..9: note = LCDR3
SQSTHVPLT

SEQ ID NO: 85 - protein, 16 aa, artificial sequence
  REGION 1..16: note = LCDR1
RSSQSLVHSSGNTYLH

SEQ ID NO: 86 - protein, 16 aa, artificial sequence
  REGION 1..16: note = LCDR1
SSSQSLVHSNGNTYLH

SEQ ID NO: 87 - protein, 16 aa, artificial sequence
  REGION 1..16: note = LCDR1
SSSQSLVHSSGNTYLH

SEQ ID NO: 88 - protein, 9 aa, artificial sequence
  REGION 1..9: note = LCDR3
SQNTHVPLT

SEQ ID NO: 89 - protein, 16 aa, artificial sequence
  REGION 1..16: note = LCDR1
KSSQSLLYSNGKTYLY

SEQ ID NO: 90 - protein, 7 aa, artificial sequence
  REGION 1..7: note = LCDR2
LVSKLDS

SEQ ID NO: 91 - protein, 9 aa, artificial sequence
  REGION 1..9: note = LCDR3
VQGTHFPYT

SEQ ID NO: 92 - protein, 16 aa, artificial sequence
  REGION 1..16: note = LCDR1
KSSQSLLYSSGKTYLY

SEQ ID NO: 93 - protein, 7 aa, artificial sequence
  REGION 1..7: note = LCDR2
LVSKLDA

SEQ ID NO: 94 - protein, 11 aa, artificial sequence
  REGION 1..11: note = LCDR1
RASQSISDYLH

SEQ ID NO: 95 - protein, 7 aa, artificial sequence
  REGION 1..7: note = LCDR2
YASQSIS

SEQ ID NO: 96 - protein, 9 aa, artificial sequence
  REGION 1..9: note = LCDR3
QNGHSFPYT

SEQ ID NO: 97 - protein, 9 aa, artificial sequence
  REGION 1..9: note = LCDR3
QSGHSFPYT

SEQ ID NO: 98 - protein, 9 aa, artificial sequence
  REGION 1..9: note = LCDR3
QNAHSFPYT

SEQ ID NO: 99 - protein, 11 aa, artificial sequence
  REGION 1..11: note = LCDR1
KASQDINSYLS

SEQ ID NO: 100 - protein, 7 aa, artificial sequence
  REGION 1..7: note = LCDR2
RANRLVD

SEQ ID NO: 101 - protein, 9 aa, artificial sequence
  REGION 1..9: note = LCDR3
LQYDEFPYT

SEQ ID NO: 102 - protein, 11 aa, artificial sequence
  REGION 1..11: note = LCDR1
KASQDITSYLS

SEQ ID NO: 103 - protein, 7 aa, artificial sequence
  REGION 1..7: note = LCDR2
RANRLVS

SEQ ID NO: 104 - protein, 329 aa, artificial sequence
  REGION 1..329: note = Heavy chain constant region
ASTKGPSVFPLAPSSKSTSGGTAALGCLVKDYFPEPVTVSWNSGALTSGVHTFPAVLQSSGLYSLSSVVTVPSSSLGTQTYICNVNHKPSNTKVDKKVEPKSCDKTHTCPPCPAPELLGGPSVFLFPPKPKDTLMISRTPEVTCVVVDVSHEDPEVKFNWYVDGVEVHNAKTKPREEQYNSTYRVVSVLTVLHQDWLNGKEYKCKVSNKALPAPIEKTISKAKGQPREPQVYTLPPSREEMTKNQVSLTCLVKGFYPSDIAVEWESNGQPENNYKTTPPVLDSDGSFFLYSKLTVDKSRWQQGNVFSCSVMHEALHNHYTQKSLSLSPG

SEQ ID NO: 105 - protein, 107 aa, artificial sequence [sequence omitted]